European Patent Specification EP 3 406 723 B1, published January 8, 2025. Title: AN IL-15 AND IL-15Ralpha SUSHI DOMAIN BASED IMMUNOCYTOKINES. Applicant: CYTUNE PHARMA INSERM (Institut National de la Santé et de la Recherche Médicale). Application Divisional application based on EP12731303.9. The sequence listing filed with the application follows.

SEQUENCE LISTING (27 sequences)

SEQ ID NO: 1 - protein, 114 aa, artificial sequence
  mammalian interleukin 15 consensus sequence
  MISC_FEATURE (1)..(1): X= N, S, T or I
  MISC_FEATURE (3)..(3): X= V, H, I, Q or E
  MISC_FEATURE (4)..(4): X= N, Y, F or D
  MISC_FEATURE (6)..(6): X= I or R
  MISC_FEATURE (7)..(7): X= S, N, L, Y, K or R
  MISC_FEATURE (10)..(10): X= K, E, R or Q
  MISC_FEATURE (11)..(11): X= K, T or R
  MISC_FEATURE (13)..(13): X= E, D or Q
  MISC_FEATURE (14)..(14): X= D, H, S or N
  MISC_FEATURE (16)..(16): X= I or T
  MISC_FEATURE (17)..(17): X=Q, R or K
  MISC_FEATURE (18)..(18): X= S or F
  MISC_FEATURE (19)..(19): X= M, I or L
  MISC_FEATURE (21)..(21): X= I, V or M
  MISC_FEATURE (23)..(23): X=A or T
  MISC_FEATURE (28)..(28): X=E or D
  MISC_FEATURE (30)..(30): X= D or G
  MISC_FEATURE (31)..(31): X= V, F, A or I
  MISC_FEATURE (34)..(34): X= S, N or R
  MISC_FEATURE (37)..(37): X= V or I
  MISC_FEATURE (39)..(39): X= A or T
  MISC_FEATURE (41)..(41): X= K, Q or N
  MISC_FEATURE (48)..(48): X= Q, G, R, H or E
  MISC_FEATURE (51)..(51): X= S or L
  MISC_FEATURE (52)..(52): X= L, Q or H
  MISC_FEATURE (54)..(54): X= S, F or Y
  MISC_FEATURE (55)..(55): X= G, K, S, N or R
  MISC_FEATURE (56)..(56): X= D, H, S or N
  MISC_FEATURE (57)..(57): X= A, H, M, E, G, S or T
  MISC_FEATURE (58)..(58): X= S, V, P, T, N or D
  MISC_FEATURE (59)..(59): X= I or L
  MISC_FEATURE (60)..(60): X=  H, S, K, N, Y or E
  MISC_FEATURE (61)..(61): X=  D or E
  MISC_FEATURE (62)..(62): X=  T, I or A
  MISC_FEATURE (63)..(63): X=  V or I
  MISC_FEATURE (64)..(64): X=  E, T, Q, R or K
  MISC_FEATURE (66)..(66): X=  L or V
  MISC_FEATURE (67)..(67): X= I, T or L
  MISC_FEATURE (68)..(68): X=I, M, F, Y or L
  MISC_FEATURE (72)..(72): X= N, T, R, D or S
  MISC_FEATURE (73)..(73): X= S, N, R, T or I
  MISC_FEATURE (75)..(75): X= S or N
  MISC_FEATURE (76)..(76): X= S or A
  MISC_FEATURE (77)..(77): X= N, I or K
  MISC_FEATURE (78)..(78): X= G, E or K
  MISC_FEATURE (79)..(79): X= N, Y, D or T
  MISC_FEATURE (80)..(80): X= V, K or I
  MISC_FEATURE (81)..(81): X= T, A or I
  MISC_FEATURE (83)..(83): X= S, L or T
  MISC_FEATURE (87)..(87): X= E or V
  MISC_FEATURE (93)..(93): X= E or K
  MISC_FEATURE (94)..(94): X= K or R
  MISC_FEATURE (95)..(95): X= N, T or S
  MISC_FEATURE (96)..(96): X= I or F
  MISC_FEATURE (97)..(97): X= K, N, A, or T
  MISC_FEATURE (101)..(101): X= Q, K or E
  MISC_FEATURE (104)..(104): X= V, I or K
  MISC_FEATURE (105)..(105): X= H or R
  MISC_FEATURE (112)..(112): X= N or Y
  MISC_FEATURE (113)..(113): X= = T, S, P, L or A
  MISC_FEATURE (114)..(114): X= = S or P
XWXXVXXDLXXIXXLXXXXHXDXTLYTXSXXHPXCKXTXMXCFLLELXVIXXEXXXXXXXXXXXNXXXLANXXLXXXXXXXEXGCKXCEELEXXXXXEFLXSFXXIVQMFIXXX

SEQ ID NO: 2 - protein, 114 aa, Artificial Sequence
  primate uinterleukin 15 consensus sequence
  MISC_FEATURE (1)..(1): X = N or I
  MISC_FEATURE (4)..(4): X = N or D
  MISC_FEATURE (10)..(10): X = K or R
  MISC_FEATURE (11)..(11): X = K or R
  MISC_FEATURE (13)..(13): X = E or Q
  MISC_FEATURE (16)..(16): X = I or T
  MISC_FEATURE (19)..(19): X = M or I
  MISC_FEATURE (30)..(30): X = D or G
  MISC_FEATURE (31)..(31): X = V or I
  MISC_FEATURE (34)..(34): X = S or R
  MISC_FEATURE (52)..(52): X = L or H
  MISC_FEATURE (55)..(55): X = G or N
  MISC_FEATURE (56)..(56): X = D or N
  MISC_FEATURE (57)..(57): X = A or T
  MISC_FEATURE (58)..(58): X = S, N or D
  MISC_FEATURE (60)..(60): X = H or N
  MISC_FEATURE (63)..(63): X = V or I
  MISC_FEATURE (67)..(67): X = I or L
  MISC_FEATURE (72)..(72): X = N or R
  MISC_FEATURE (73)..(73): X =S or I
  MISC_FEATURE (76)..(76): X =S or A
  MISC_FEATURE (79)..(79): X =N or T
  MISC_FEATURE (80)..(80): X =V or I
  MISC_FEATURE (93)..(93): X =E or K
  MISC_FEATURE (112)..(112): X = N or Y
  MISC_FEATURE (113)..(113): X = T or A
XWVXVISDLXXIXDLXQSXHIDATLYTESXXHPXCKVTAMKCFLLELQVISXESXXXXIXDTXENLXILANXXLSXNGXXTESGCKECEELEXKNIKEFLQSFVHIVQMFIXXS

SEQ ID NO: 3 - protein, 114 aa, Homo sapiens
  VARIANT (93)..(93): X= E or K
NWVNVISDLKKIEDLIQSMHIDATLYTESDVHPSCKVTAMKCFLLELQVISLESGDASIHDTVENLIILANNSLSSNGNVTESGCKECEELEXKNIKEFLQSFVHIVQMFINTS

SEQ ID NO: 4 - protein, 61 aa, Artificial Sequence
  mammalian sushi domain consensus sequence
  MISC_FEATURE (3)..(3): X= P or A
  MISC_FEATURE (5)..(5): X= M or V
  MISC_FEATURE (7)..(7): X= V or I
  MISC_FEATURE (13)..(13): X= W, R or Q
  MISC_FEATURE (16)..(16): X= S or N
  MISC_FEATURE (19)..(19): X= L or V
  MISC_FEATURE (20)..(20): X= Y, H or N
  MISC_FEATURE (26)..(26): X= I or V
  MISC_FEATURE (39)..(39): X= S or T
  MISC_FEATURE (41)..(41): X=T or I
  MISC_FEATURE (45)..(45): X=T or I
  MISC_FEATURE (45)..(45): X= L or I
  MISC_FEATURE (48)..(48): X= A or N
  MISC_FEATURE (51)..(51): X= V or A
  MISC_FEATURE (53)..(53): X= H or Y
CPXPXSXEHADIXVKXYSXXSRERYXCNSGFKRKAGTSXLXECVXNKXTNXAXWTTPSLKC

SEQ ID NO: 5 - protein, 64 aa, Artificial Sequence
  enlarged mammalian sushi domain consensus sequence
  MISC_FEATURE (1)..(1): X= T, V or I
  MISC_FEATURE (5)..(5): X= P or A
  MISC_FEATURE (7)..(7): X= M or V
  MISC_FEATURE (9)..(9): X= V or I
  MISC_FEATURE (15)..(15): X= W, R or Q
  MISC_FEATURE (18)..(18): X= S or N
  MISC_FEATURE (21)..(21): X=L or V
  MISC_FEATURE (22)..(22): X=Y, H or N
  MISC_FEATURE (28)..(28): X= I or V
  MISC_FEATURE (41)..(41): X= S or T
  MISC_FEATURE (43)..(43): X= T or I
  MISC_FEATURE (47)..(47): X= L or I
  MISC_FEATURE (50)..(50): X= A or N
  MISC_FEATURE (53)..(53): X= V or A
  MISC_FEATURE (55)..(55): X= H or Y
XTCPXPXSXEHADIXVKXYSXXSRERYXCNSGFKRKAGTSXLXECVXNKXTNXAXWTTPSLKCI

SEQ ID NO: 6 - protein, 61 aa, Artificial Sequence
  primate sushi domain consensus sequence
  MISC_FEATURE (3)..(3): X= P or A
  MISC_FEATURE (5)..(5): X= M or V
  MISC_FEATURE (13)..(13): X= W, R or Q
  MISC_FEATURE (20)..(20): X= Y or H
  MISC_FEATURE (26)..(26): X= I or V
  MISC_FEATURE (51)..(51): X= V or A
  MISC_FEATURE (53)..(53): X= V or A
CPXPXSVEHADIXVKSYSLXSRERYXCNSGFKRKAGTSSLTECVLNKATNXAXWTTPSLKC

SEQ ID NO: 7 - protein, 63 aa, Artificial Sequence
  enlarged primate sushi domain consensus sequence
  MISC_FEATURE (1)..(1): X= V or I
  MISC_FEATURE (5)..(5): X= P or A
  MISC_FEATURE (7)..(7): X= M or V
  MISC_FEATURE (15)..(15): X= W, R or Q
  MISC_FEATURE (22)..(22): X= Y or H
  MISC_FEATURE (28)..(28): X= I or V
  MISC_FEATURE (53)..(53): X=V or A
  MISC_FEATURE (55)..(55): X=H or Y
XTCPXPXSVEHADIXVKSYSLXSRERYXCNSGFKRKAGTSSLTECVLNKATNXAXWTTPSLKC

SEQ ID NO: 8 - protein, 61 aa, Homo sapiens
CPPPMSVEHADIWVKSYSLYSRERYICNSGFKRKAGTSSLTECVLNKATNVAHWTTPSLKC

SEQ ID NO: 9 - protein, 64 aa, Homo sapiens
ITCPPPMSVEHADIWVKSYSLYSRERYICNSGFKRKAGTSSLTECVLNKATNVAHWTTPSLKCI

SEQ ID NO: 10 - protein, 77 aa, Artificial Sequence
  mammalian sushi and domains consensus sequence
  MISC_FEATURE (1)..(1): X= T, V or I
  MISC_FEATURE (5)..(5): X= P or A
  MISC_FEATURE (7)..(7): X= M or V
  MISC_FEATURE (9)..(9): X= V or I
  MISC_FEATURE (15)..(15): X= W, R or Q
  MISC_FEATURE (18)..(18): X= S or N
  MISC_FEATURE (21)..(21): X= L or V
  MISC_FEATURE (22)..(22): X= Y, H or N
  MISC_FEATURE (28)..(28): X= I or V
  MISC_FEATURE (41)..(41): X= S or T
  MISC_FEATURE (43)..(43): X= T or I
  MISC_FEATURE (47)..(47): X= L or I
  MISC_FEATURE (50)..(50): X=A or N
  MISC_FEATURE (53)..(53): X= V or A
  MISC_FEATURE (55)..(55): X= H or Y
  MISC_FEATURE (55)..(55): X= H or Y
  MISC_FEATURE (68)..(68): X=A, S or L
  MISC_FEATURE (70)..(70): X= V, A, S or T
  MISC_FEATURE (71)..(71): X= H or R
  MISC_FEATURE (72)..(72): X= Q or H
  MISC_FEATURE (73)..(73): X= R, S or K
  MISC_FEATURE (75)..(75): X= A, V or P
  MISC_FEATURE (76)..(76): X= P or S
  MISC_FEATURE (77)..(77): X= P or T
XTCPXPXSXEHADIXVKXYSXXSRERYXCNSGFKRKAGTSXLXECVXNKXTNXAXWTTPSLKCIRDPXLXXXXPXXX

SEQ ID NO: 11 - protein, 77 aa, Artificial Sequence
  primate sushi and domains consensus sequence
  MISC_FEATURE (1)..(1): X= V or I
  MISC_FEATURE (5)..(5): X= P or A
  MISC_FEATURE (7)..(7): X= M or V
  MISC_FEATURE (15)..(15): X= W, R or Q
  MISC_FEATURE (22)..(22): X= Y or H
  MISC_FEATURE (28)..(28): X= I or V
  MISC_FEATURE (53)..(53): X= V or A
  MISC_FEATURE (55)..(55): X= H or Y
  MISC_FEATURE (68)..(68): X= A, S or L
  MISC_FEATURE (70)..(70): X= V, A or T
  MISC_FEATURE (71)..(71): X= H or R
  MISC_FEATURE (75)..(75): X= A or V
XTCPXPXSVEHADIXVKSYSLXSRERYXCNSGFKRKAGTSSLTECVLNKATNXAXWTTPSLKCIRDPXLXXQRPXPP

SEQ ID NO: 12 - protein, 77 aa, Homo sapiens
ITCPPPMSVEHADIWVKSYSLYSRERYICNSGFKRKAGTSSLTECVLNKATNVAHWTTPSLKCIRDPALVHQRPAPP

SEQ ID NO: 13 - protein, 20 aa, Artificial Sequence
  peptidic linker
SGGSGGGGSGGGSGGGGSLQ

SEQ ID NO: 14 - protein, 20 aa, Artificial Sequence
  peptidic linker
SGGSGGGGSGGGSGGGGSGG

SEQ ID NO: 15 - protein, 21 aa, Artificial Sequence
  peptidic linker
SGGGSGGGGSGGGGSGGGSLQ

SEQ ID NO: 16 - protein, 22 aa, Artificial Sequence
  peptidic linker
SGGGGSGGGGSGGGGSGGGGSG

SEQ ID NO: 17 - protein, 211 aa, Artificial Sequence
  RLI
ITCPPPMSVEHADIWVKSYSLYSRERYICNSGFKRKAGTSSLTECVLNKATNVAHWTTPSLKCIRDPALVHQRPAPPSGGSGGGGSGGGSGGGGSGGNWVNVISDLKKIEDLIQSMHIDATLYTESDVHPSCKVTAMKCFLLELQVISLESGDASIHDTVENLIILANNSLSSNGNVTESGCKECEELEEKNIKEFLQSFVHIVQMFINTS

SEQ ID NO: 18 - protein, 234 aa, Artificial Sequence
  ANti-HER2Neu light chain
MARSVTLVFLVLVSLTGLYADIVMTQSHKFMSTSVGDRVSITCKASQDVNTAVAWYQQKPGHSPKLLIYSASFRYTGVPDRFTGNRSGTDFTFTISSVQAEDLAVYYCQQHYTTPPTFGGGTKVEIKRADAAPTVSIFPPSSEQLTSGGASVVCFLNNFYPKDINVKWKIDGSERQNGVLNSWTDQDSKDSTYSMSSTLTLTKDEYERHNSYTCEATHKTSTSPIVKSFNRNEC

SEQ ID NO: 19 - protein, 464 aa, Artificial Sequence
  Anti-HER2Neu heavy chain
MARSVTLVFLVLVSLTGLYAQVQLQQSGPELVKPGASLKLSCTASGFNIKDTYIHWVKQRPEQGLEWIGRIYPTNGYTRYDPKFQDKATITADTSSNTAYLQVSRLTSEDTAVYYCSRWGGDGFYAMDYWGQGASVTVSSAKTTPPSVYPLAPGSAAQTNSMVTLGCLVKGYFPEPVTVTWNSGSLSSGVHTFPAVLQSDLYTLSSSVTVPSSTWPSETVTCNVAHPASSTKVDKKIVPRDCGCKPCICTVPEVSSVFIFPPKPKDVLTITLTPKVTCVVVDISKDDPEVQFSWFVDDVEVHTAQTQPREEQFNSTFRSVSELPIMHQDWLNGKEFKCRVNSAAFPAPIEKTISKTKGRPKAPQVYTIPPPKEQMAKDKVSLTCMITDFFPEDITVEWQWNGQPAENYKNTQPIMDTDGSYFVYSKLNVQKSNWEAGNTFTCSVLHEGLHNHHTEKSLSHSPGK

SEQ ID NO: 20 - protein, 600 aa, Artificial Sequence
  IL15-L22-anti HER2Neu heavy chain
MARSVTLVFLVLVSLTGLYAQVQLQQSGPELVKPGASLKLSCTASGFNIKDTYIHWVKQRPEQGLEWIGRIYPTNGYTRYDPKFQDKATITADTSSNTAYLQVSRLTSEDTAVYYCSRWGGDGFYAMDYWGQGASVTVSSAKTTPPSVYPLAPGSAAQTNSMVTLGCLVKGYFPEPVTVTWNSGSLSSGVHTFPAVLQSDLYTLSSSVTVPSSTWPSETVTCNVAHPASSTKVDKKIVPRDCGCKPCICTVPEVSSVFIFPPKPKDVLTITLTPKVTCVVVDISKDDPEVQFSWFVDDVEVHTAQTQPREEQFNSTFRSVSELPIMHQDWLNGKEFKCRVNSAAFPAPIEKTISKTKGRPKAPQVYTIPPPKEQMAKDKVSLTCMITDFFPEDITVEWQWNGQPAENYKNTQPIMDTDGSYFVYSKLNVQKSNWEAGNTFTCSVLHEGLHNHHTEKSLSHSPGKSGGGGSGGGGSGGGGSGGGGSGNWVNVISDLKKIEDLIQSMHIDATLYTESDVHPSCKVTAMKCFLLELQVISLESGDASIHDTVENLIILANNSLSSNGNVTESGCKECEELEEKNIKEFLQSFVHIVQMFINTS

SEQ ID NO: 21 - protein, 578 aa, Artificial Sequence
  IL15-anti HER2Neu Heavy chain
MARSVTLVFLVLVSLTGLYAQVQLQQSGPELVKPGASLKLSCTASGFNIKDTYIHWVKQRPEQGLEWIGRIYPTNGYTRYDPKFQDKATITADTSSNTAYLQVSRLTSEDTAVYYCSRWGGDGFYAMDYWGQGASVTVSSAKTTPPSVYPLAPGSAAQTNSMVTLGCLVKGYFPEPVTVTWNSGSLSSGVHTFPAVLQSDLYTLSSSVTVPSSTWPSETVTCNVAHPASSTKVDKKIVPRDCGCKPCICTVPEVSSVFIFPPKPKDVLTITLTPKVTCVVVDISKDDPEVQFSWFVDDVEVHTAQTQPREEQFNSTFRSVSELPIMHQDWLNGKEFKCRVNSAAFPAPIEKTISKTKGRPKAPQVYTIPPPKEQMAKDKVSLTCMITDFFPEDITVEWQWNGQPAENYKNTQPIMDTDGSYFVYSKLNVQKSNWEAGNTFTCSVLHEGLHNHHTEKSLSHSPGKNWVNVISDLKKIEDLIQSMHIDATLYTESDVHPSCKVTAMKCFLLELQVISLESGDASIHDTVENLIILANNSLSSNGNVTESGCKECEELEEKNIKEFLQSFVHIVQMFINTS

SEQ ID NO: 22 - protein, 697 aa, Artificial Sequence
  ELI-L22-anti HER2Neu Heavy Chain
MARSVTLVFLVLVSLTGLYAQVQLQQSGPELVKPGASLKLSCTASGFNIKDTYIHWVKQRPEQGLEWIGRIYPTNGYTRYDPKFQDKATITADTSSNTAYLQVSRLTSEDTAVYYCSRWGGDGFYAMDYWGQGASVTVSSAKTTPPSVYPLAPGSAAQTNSMVTLGCLVKGYFPEPVTVTWNSGSLSSGVHTFPAVLQSDLYTLSSSVTVPSSTWPSETVTCNVAHPASSTKVDKKIVPRDCGCKPCICTVPEVSSVFIFPPKPKDVLTITLTPKVTCVVVDISKDDPEVQFSWFVDDVEVHTAQTQPREEQFNSTFRSVSELPIMHQDWLNGKEFKCRVNSAAFPAPIEKTISKTKGRPKAPQVYTIPPPKEQMAKDKVSLTCMITDFFPEDITVEWQWNGQPAENYKNTQPIMDTDGSYFVYSKLNVQKSNWEAGNTFTCSVLHEGLHNHHTEKSLSHSPGKSGGGGSGGGGSGGGGSGGGGSGITCPPPMSVEHADIWVKSYSLYSRERYICNSGFKRKAGTSSLTECVLNKATNVAHWTTPSLKCIRDPALVHQRPAPPSGGSGGGGSGGGSGGGGSGGNWVNVISDLKKIEDLIQSMHIDATLYTESDVHPSCKVTAMKCFLLELQVISLESGDASIHDTVENLIILANNSLSSNGNVTESGCKECEELEEKNIKEFLQSFVHIVQMFINTS

SEQ ID NO: 23 - protein, 675 aa, Artificial Sequence
  RLI-anti HER2Neu Heavy chain
MARSVTLVFLVLVSLTGLYAQVQLQQSGPELVKPGASLKLSCTASGFNIKDTYIHWVKQRPEQGLEWIGRIYPTNGYTRYDPKFQDKATITADTSSNTAYLQVSRLTSEDTAVYYCSRWGGDGFYAMDYWGQGASVTVSSAKTTPPSVYPLAPGSAAQTNSMVTLGCLVKGYFPEPVTVTWNSGSLSSGVHTFPAVLQSDLYTLSSSVTVPSSTWPSETVTCNVAHPASSTKVDKKIVPRDCGCKPCICTVPEVSSVFIFPPKPKDVLTITLTPKVTCVVVDISKDDPEVQFSWFVDDVEVHTAQTQPREEQFNSTFRSVSELPIMHQDWLNGKEFKCRVNSAAFPAPIEKTISKTKGRPKAPQVYTIPPPKEQMAKDKVSLTCMITDFFPEDITVEWQWNGQPAENYKNTQPIMDTDGSYFVYSKLNVQKSNWEAGNTFTCSVLHEGLHNHHTEKSLSHSPGKITCPPPMSVEHADIWVKSYSLYSRERYICNSGFKRKAGTSSLTECVLNKATNVAHWTTPSLKCIRDPALVHQRPAPPSGGSGGGGSGGGSGGGGSGGNWVNVISDLKKIEDLIQSMHIDATLYTESDVHPSCKVTAMKCFLLELQVISLESGDASIHDTVENLIILANNSLSSNGNVTESGCKECEELEEKNIKEFLQSFVHIVQMFINTS

SEQ ID NO: 24 - protein, 427 aa, Artificial Sequence
  IL15-L22-ScFv fragment HER2Neu
MARSVTLVFLVLVSLTGLYADIVMTQSPSSLSASVGDRVTITCRASQDVNTAVAWYQQKPGKAPKLLIYSASFLYSGVPSRFSGSRSGTDFTLTISSLQPEDFATYYCQQHYTTPPTFGQGTKVELKRATPSHNSHQVPSAGGPTANSGEVKLVESGGGLVQPGGSLRLSCATSGFNIKDTYIHWVRQAPGKGLEWVARIYPTNGYTRYADSVKGRFTISADTSKNTAYLQMNSLRAEDTAVYYCSRWGGDGFYAMDYWGQGTTVTVSSGGGGSGGGGSGGGGSGGGGSGNWVNVISDLKKIEDLIQSMHIDATLYTESDVHPSCKVTAMKCFLLELQVISLESGDASIHDTVENLIILANNSLSSNGNVTESGCKECEELEEKNIKEFLQSFVHIVQMFINTSEEKNIKEFLQSFVHIVQMFINTS

SEQ ID NO: 25 - protein, 405 aa, Artificial Sequence
  IL15-ScFv fragment HER2Neu
MARSVTLVFLVLVSLTGLYADIVMTQSPSSLSASVGDRVTITCRASQDVNTAVAWYQQKPGKAPKLLIYSASFLYSGVPSRFSGSRSGTDFTLTISSLQPEDFATYYCQQHYTTPPTFGQGTKVELKRATPSHNSHQVPSAGGPTANSGEVKLVESGGGLVQPGGSLRLSCATSGFNIKDTYIHWVRQAPGKGLEWVARIYPTNGYTRYADSVKGRFTISADTSKNTAYLQMNSLRAEDTAVYYCSRWGGDGFYAMDYWGQGTTVTVSNWVNVISDLKKIEDLIQSMHIDATLYTESDVHPSCKVTAMKCFLLELQVISLESGDASIHDTVENLIILANNSLSSNGNVTESGCKECEELEEKNIKEFLQSFVHIVQMFINTSEEKNIKEFLQSFVHIVQMFINTS

SEQ ID NO: 26 - protein, 501 aa, Artificial Sequence [sequence omitted]

SEQ ID NO: 27 - protein, 479 aa, Artificial Sequence
  RLI-ScFv fragment HER2Neu frgament
MARSVTLVFLVLVSLTGLYADIVMTQSPSSLSASVGDRVTITCRASQDVNTAVAWYQQKPGKAPKLLIYSASFLYSGVPSRFSGSRSGTDFTLTISSLQPEDFATYYCQQHYTTPPTFGQGTKVELKRATPSHNSHQVPSAGGPTANSGEVKLVESGGGLVQPGGSLRLSCATSGFNIKDTYIHWVRQAPGKGLEWVARIYPTNGYTRYADSVKGRFTISADTSKNTAYLQMNSLRAEDTAVYYCSRWGGDGFYAMDYWGQGTTVTVSITCPPPMSVEHADIWVKSYSLYSRERYICNSGFKRKAGTSSLTECVLNKATNVAHWTTPSLKCIRDPALVHQRPAPPSGGSGGGGSGGGSGGGGSGGNWVNVISDLKKIEDLIQSMHIDATLYTESDVHPSCKVTAMKCFLLELQVISLESGDASIHDTVENLIILANNSLSSNGNVTESGCKECEELEEKNIKEFLQSFVHIVQMFINTS